European Patent Application EP 4 331 609 A1, published March 6, 2024. Title: Composition for an enhanced delivery of a polyplex. Applicant: Sapreme Technologies B.V. Application EP, filed September 1, 2022. The sequence listing filed with the application follows.

SEQUENCE LISTING (2 sequences)

SEQ ID NO: 1 - protein, 24 aa, synthetic construct
KKKKKKKKKKKKKKKKGGGGCGGY

SEQ ID NO: 2 - protein, 25 aa, synthetic construct
KKKKKKKKKKKKKKKKGGGGCGGYK